European Patent Specification EP 3 320 116 B1, published August 30, 2023. Title: METHODS FOR DIAGNOSING BLADDER CANCER. Applicant: Nucleix Ltd. The sequence listing filed with the application follows.

SEQUENCE LISTING (167 sequences)

SEQ ID NO: 1 - DNA, 60 bp, Homo sapiens
tttttaggggtctgcgcgctctcgcctggctgctgggaaggagggctgggaggcgctgaa

SEQ ID NO: 2 - DNA, 140 bp, Homo sapiens
tccaggcgcgccgaccgctcaagcgctccaggtccacccggcggagggcagagaaagcgcgaccgcgcggcccgcagggttgcaagaagaaaacgagtgttatataatgagtctcagtggttgctcacaatgccaggcgc

SEQ ID NO: 3 - DNA, 60 bp, Homo sapiens
ggctgataccagagaggacccggagcgcgaaccagaggttcgacctccagggcagcgcag

SEQ ID NO: 4 - DNA, 130 bp, Homo sapiens
ggggcgccaaatgcccacgtgttgatgaaaccagtgagatgggaacaggcggcgggaaaccagacagaggaagagctagggaggagaccccagccccggatcctgggtcgccagggttttccgcgcgcat

SEQ ID NO: 5 - DNA, 70 bp, Homo sapiens
tctgagaagtgtcctcctcgctctcttataaaaacaggacttgttgccgaggtcagcgcgcgcatcgagt

SEQ ID NO: 6 - DNA, 130 bp, Homo sapiens
atcagcgcgaactattcgtttagtggccttaaaacaccctggtttcaccctcagctattttcaagttcccgtgtgcctggcactttctccgtgcgagaagcaccggagggtgcggacgcgccacagtctg

SEQ ID NO: 7 - DNA, 150 bp, Homo sapiens
tgctctgcgcagcgtggagggcaacgggactgggaggcggcttctgccgccgggcactcgcttccaggtggcttacgaggattcagactgtgggaaccgtgcgctcttcagcttggtggaccgcgtggcggcggcgcggggcgccaagcc

SEQ ID NO: 8 - DNA, 70 bp, Homo sapiens
cgcgcagaactttgcggtggcgcttagcgcctcctttgcccagacccttcccgcctttgccgcgcccaga

SEQ ID NO: 9 - DNA, 70 bp, Homo sapiens
cgtaatcgccggtgtaactcatgttggctggggggcctcccggcgcgcgcggagaggctggggtgcgccc

SEQ ID NO: 10 - DNA, 60 bp, Homo sapiens
cgattcagagggccccggtcggagctgtcggagattgagcgcgcgcggtcccgggatctc

SEQ ID NO: 11 - DNA, 140 bp, Homo sapiens
cgcgcggcagccctccgtgcgcgcaggctcgggtgcgttgttcgcgggggtgaattgtgaagaaccatcgcggggtccttcctgctgaggccgcggacaccgtgacctcgctgctctgggtctgcagggaaacgtaggaa

SEQ ID NO: 12 - DNA, 100 bp, Homo sapiens
tgacctttaggggctgttactctcagaccaggcccagcagcacccggcgcatttacgtcggatctgacccctgcaagcaccggcgcgaccgcgctagcgg

SEQ ID NO: 13 - DNA, 70 bp, Homo sapiens
agaacttcgtgggcaggtaagcgcgcagggcgcggagtaaggatgcggcagtggggcgaccccgctgcgg

SEQ ID NO: 14 - DNA, 70 bp, Homo sapiens
ctgcctgcgctcactacgggttttttagttggcgccttaatgtttgtaacacttttagagcgcttgctct

SEQ ID NO: 15 - DNA, 140 bp, Homo sapiens
ggccgggaagcgcggggtgagaaagcgaggtgggtggcgagagcgtgagcgcccctctgctgaccccggggagcgtggactacgagttggcgcccaagtccagaatccgcgcgcaccgcggtaagctgcgccttttgaaa

SEQ ID NO: 16 - DNA, 60 bp, Homo sapiens
agactaacttttctcttgtacagaatcatcaggctaaatttttggcattatttcagtcct

SEQ ID NO: 17 - DNA, 80 bp, Artificial Sequence
  Control construct
aagtctcgagtcgatgtcactaaccatgagtattccatgtgccgtcatctaacaagtactgcataccctggataatggct

SEQ ID NO: 18 - DNA, 100 bp, Artificial Sequence
  Control construct
taccaggtctacaaagctcgactctgcctgcgctcactacgggttttttagttggcgccttaatgtttgtaacacttttagagcgcttgctctgatcctc

SEQ ID NO: 19 - DNA, 20 bp, Artificial Sequence
  Primer
aagtctcgagtcgatgtcac

SEQ ID NO: 20 - DNA, 20 bp, Artificial Sequence
  Primer
agccattatccagggtatgc

SEQ ID NO: 21 - DNA, 23 bp, Artificial Sequence
  Probe
accatgagtattccatgtgccgt

SEQ ID NO: 22 - DNA, 22 bp, Artificial Sequence
  Primer
taccaggtctacaaagctcgac

SEQ ID NO: 23 - DNA, 23 bp, Artificial Sequence
  Primer
acgcctactaatacacatcggag

SEQ ID NO: 24 - DNA, 25 bp, Artificial Sequence
  Probe
cgctcactacgggttttttagttgg

SEQ ID NO: 25 - DNA, 21 bp, Artificial Sequence
  Primer
cagacccggttaacactgaag

SEQ ID NO: 26 - DNA, 23 bp, Artificial Sequence
  Primer
gacccggttaacactgaagttgc

SEQ ID NO: 27 - DNA, 20 bp, Artificial Sequence
  Primer
ccagacccggttaacactga

SEQ ID NO: 28 - DNA, 22 bp, Artificial Sequence
  Primer
ccggttaacactgaagttgctt

SEQ ID NO: 29 - DNA, 21 bp, Artificial Sequence
  Primer
tccagacccggttaacactga

SEQ ID NO: 30 - DNA, 20 bp, Artificial Sequence
  Primer
ctcagatctgccctcgcttc

SEQ ID NO: 31 - DNA, 20 bp, Artificial Sequence
  Primer
ctcagatctgccctcgcttc

SEQ ID NO: 32 - DNA, 23 bp, Artificial Sequence
  Primer
gcaactcctacagacactcagat

SEQ ID NO: 33 - DNA, 20 bp, Artificial Sequence
  Primer
gacactcagatctgccctcg

SEQ ID NO: 34 - DNA, 25 bp, Artificial Sequence
  Primer
atcagaacaattagagagtaatgat

SEQ ID NO: 35 - DNA, 19 bp, Artificial Sequence
  Primer
cagatctgccctcgcttca

SEQ ID NO: 36 - DNA, 20 bp, Artificial Sequence
  Primer
ggtccagcagctagtccact

SEQ ID NO: 37 - DNA, 20 bp, Artificial Sequence
  Primer
ctccctggtccagcagctag

SEQ ID NO: 38 - DNA, 18 bp, Artificial Sequence
  Primer
cccgcctggctgctccag

SEQ ID NO: 39 - DNA, 21 bp, Artificial Sequence
  Primer
caccaggtgcaaaagatgcct

SEQ ID NO: 40 - DNA, 20 bp, Artificial Sequence
  Primer
cgggaagggaaaggccacat

SEQ ID NO: 41 - DNA, 21 bp, Artificial Sequence
  Primer
aaggccacatcttcacgcctt

SEQ ID NO: 42 - DNA, 22 bp, Artificial Sequence
  Primer
tgagcaaccactgagactcatt

SEQ ID NO: 43 - DNA, 19 bp, Artificial Sequence
  Primer
cgtcctggagctccgactc

SEQ ID NO: 44 - DNA, 19 bp, Artificial Sequence
  Primer
ccgactcccaccccatctg

SEQ ID NO: 45 - DNA, 20 bp, Artificial Sequence
  Primer
ataccagagaggacccggag

SEQ ID NO: 46 - DNA, 21 bp, Artificial Sequence
  Primer
gaaccagaggttcgacctcca

SEQ ID NO: 47 - DNA, 19 bp, Artificial Sequence
  Primer
cccggcttcggagcgggaa

SEQ ID NO: 48 - DNA, 21 bp, Artificial Sequence
  Primer
cagtttcaccgctcgatcttg

SEQ ID NO: 49 - DNA, 20 bp, Artificial Sequence
  Primer
cgagtccagggcgaggtaag

SEQ ID NO: 50 - DNA, 21 bp, Artificial Sequence
  Primer
gaggctgataccagagaggac

SEQ ID NO: 51 - DNA, 21 bp, Artificial Sequence
  Primer
cacaactgcctgcgagaaaca

SEQ ID NO: 52 - DNA, 19 bp, Artificial Sequence
  Primer
agcttgtggcgaccccgtc

SEQ ID NO: 53 - DNA, 21 bp, Artificial Sequence
  Primer
tagctcatcccgtccagcttg

SEQ ID NO: 54 - DNA, 19 bp, Artificial Sequence
  Primer
cgcctcagccactcctggg

SEQ ID NO: 55 - DNA, 20 bp, Artificial Sequence
  Primer
ggccttggagcccaaaccag

SEQ ID NO: 56 - DNA, 19 bp, Artificial Sequence
  Primer
gctcgggcagagccaagga

SEQ ID NO: 57 - DNA, 20 bp, Artificial Sequence
  Primer
tcttgtgtgggtgccttgga

SEQ ID NO: 58 - DNA, 22 bp, Artificial Sequence
  Primer
ctggaggtcgaacctctggttc

SEQ ID NO: 59 - DNA, 19 bp, Artificial Sequence
  Primer
cgctccgaagccggggtac

SEQ ID NO: 60 - DNA, 20 bp, Artificial Sequence
  Primer
ggtgggagtcggagctccag

SEQ ID NO: 61 - DNA, 20 bp, Artificial Sequence
  Primer
ggagcgacccaaatgtggag

SEQ ID NO: 62 - DNA, 22 bp, Artificial Sequence
  Primer
cctgggcatcgtttacatttgg

SEQ ID NO: 63 - DNA, 20 bp, Artificial Sequence
  Primer
gcatcgtttacatttggggc

SEQ ID NO: 64 - DNA, 21 bp, Artificial Sequence
  Primer
gagtagagcaccaagatagtg

SEQ ID NO: 65 - DNA, 20 bp, Artificial Sequence
  Primer
gcagccgcaccttttgggat

SEQ ID NO: 66 - DNA, 20 bp, Artificial Sequence
  Primer
gggatgggatggtttggaga

SEQ ID NO: 67 - DNA, 23 bp, Artificial Sequence
  Primer
gagtctaacaaactaacctgatg

SEQ ID NO: 68 - DNA, 21 bp, Artificial Sequence
  Primer
acaggacttgttgccgaggtc

SEQ ID NO: 69 - DNA, 23 bp, Artificial Sequence
  Primer
atggacggaaataagcaaaagca

SEQ ID NO: 70 - DNA, 22 bp, Artificial Sequence
  Primer
gcaaaagcaaaacaaccccttc

SEQ ID NO: 71 - DNA, 22 bp, Artificial Sequence
  Primer
ttccgtgaaagcaatgacacag

SEQ ID NO: 72 - DNA, 22 bp, Artificial Sequence
  Primer
aataaaacaaccgctgccgaca

SEQ ID NO: 73 - DNA, 21 bp, Artificial Sequence
  Primer
caatgacacagcagaaaccac

SEQ ID NO: 74 - DNA, 20 bp, Artificial Sequence
  Primer
gccaggcactcgctggatct

SEQ ID NO: 75 - DNA, 21 bp, Artificial Sequence
  Primer
ccgccatcgataacagatcag

SEQ ID NO: 76 - DNA, 20 bp, Artificial Sequence
  Primer
ggcaccgccatcgataacag

SEQ ID NO: 77 - DNA, 21 bp, Artificial Sequence
  Primer
cccctaaacttagccagttcg

SEQ ID NO: 78 - DNA, 24 bp, Artificial Sequence
  Primer
tggcaggaacatgaataataaatg

SEQ ID NO: 79 - DNA, 19 bp, Artificial Sequence
  Primer
ggcggcggctcagactgtg

SEQ ID NO: 80 - DNA, 21 bp, Artificial Sequence
  Primer
ggcttacgaggattcagactg

SEQ ID NO: 81 - DNA, 19 bp, Artificial Sequence
  Primer
ggactgggaggcggcttct

SEQ ID NO: 82 - DNA, 19 bp, Artificial Sequence
  Primer
cgtggagggcaacgggact

SEQ ID NO: 83 - DNA, 20 bp, Artificial Sequence
  Primer
cactcgcttccaggtggctt

SEQ ID NO: 84 - DNA, 20 bp, Artificial Sequence
  Primer
cggccatcgagtatgctctg

SEQ ID NO: 85 - DNA, 23 bp, Artificial Sequence
  Primer
gatgactcgtacttgttttcact

SEQ ID NO: 86 - DNA, 21 bp, Artificial Sequence
  Primer
cccaggataaggtctggcttg

SEQ ID NO: 87 - DNA, 21 bp, Artificial Sequence
  Primer
ctgctgcatactcgcacactg

SEQ ID NO: 88 - DNA, 20 bp, Artificial Sequence
  Primer
cacactggccccaggataag

SEQ ID NO: 89 - DNA, 19 bp, Artificial Sequence
  Primer
gatgcaagccgggccactg

SEQ ID NO: 90 - DNA, 21 bp, Artificial Sequence
  Primer
ggtgatgccctgaatgttgtc

SEQ ID NO: 91 - DNA, 19 bp, Artificial Sequence
  Primer
cttaacgcctccacgccgt

SEQ ID NO: 92 - DNA, 18 bp, Artificial Sequence
  Primer
ccgtgccaggcgtcggat

SEQ ID NO: 93 - DNA, 24 bp, Artificial Sequence
  Primer
tttgtttagtacaagacatgtctg

SEQ ID NO: 94 - DNA, 23 bp, Artificial Sequence
  Primer
cgtgttgcattttgtttagtaca

SEQ ID NO: 95 - DNA, 19 bp, Artificial Sequence
  Primer
gctgcgaggcttgccgtgt

SEQ ID NO: 96 - DNA, 21 bp, Artificial Sequence
  Primer
actcggtgttctcaccgaaag

SEQ ID NO: 97 - DNA, 21 bp, Artificial Sequence
  Primer
acgtaatcgccggtgtaactc

SEQ ID NO: 98 - DNA, 22 bp, Artificial Sequence
  Primer
cctttctttgtagccacctcag

SEQ ID NO: 99 - DNA, 21 bp, Artificial Sequence
  Primer
ggaagcaacagatcgtcactc

SEQ ID NO: 100 - DNA, 22 bp, Artificial Sequence
  Primer
ttgagcacaagcatgctgcatg

SEQ ID NO: 101 - DNA, 20 bp, Artificial Sequence
  Primer
ccctctgcacactcgagaac

SEQ ID NO: 102 - DNA, 21 bp, Artificial Sequence
  Primer
ggacgagagttgagctctcac

SEQ ID NO: 103 - DNA, 21 bp, Artificial Sequence
  Primer
aggttgcagtgagccggaatg

SEQ ID NO: 104 - DNA, 25 bp, Artificial Sequence
  Primer
aataccatatagtgaacacctaaga

SEQ ID NO: 105 - DNA, 24 bp, Artificial Sequence
  Primer
ccaatttttgtgtttttagtagag

SEQ ID NO: 106 - DNA, 20 bp, Artificial Sequence
  Primer
ggatccagggcgattcagag

SEQ ID NO: 107 - DNA, 19 bp, Artificial Sequence
  Primer
cagggcctcgtcggagatc

SEQ ID NO: 108 - DNA, 19 bp, Artificial Sequence
  Primer
tcgtcggagatcccgggac

SEQ ID NO: 109 - DNA, 21 bp, Artificial Sequence
  Primer
tgctgcccagcttcttccaca

SEQ ID NO: 110 - DNA, 17 bp, Artificial Sequence
  Primer
ggtcccgcggcctccag

SEQ ID NO: 111 - DNA, 17 bp, Artificial Sequence
  Primer
gcagcttcgccgcccgg

SEQ ID NO: 112 - DNA, 18 bp, Artificial Sequence
  Primer
cggaccggccaggggtcc

SEQ ID NO: 113 - DNA, 20 bp, Artificial Sequence
  Primer
caggacccgctcagttccac

SEQ ID NO: 114 - DNA, 19 bp, Artificial Sequence
  Primer
cagggatgtgagtgggcgg

SEQ ID NO: 115 - DNA, 20 bp, Artificial Sequence
  Primer
gaagagggccgcaaaccaac

SEQ ID NO: 116 - DNA, 19 bp, Artificial Sequence
  Primer
acccgccgcactgacaggt

SEQ ID NO: 117 - DNA, 22 bp, Artificial Sequence
  Primer
tttcctacgtttccctgcagac

SEQ ID NO: 118 - DNA, 20 bp, Artificial Sequence
  Primer
atcctgcccgctcctgacaa

SEQ ID NO: 119 - DNA, 20 bp, Artificial Sequence
  Primer
ccagcaccaggagcgtgttc

SEQ ID NO: 120 - DNA, 22 bp, Artificial Sequence
  Primer
cgcgatggttcttcacaattca

SEQ ID NO: 121 - DNA, 21 bp, Artificial Sequence
  Primer
acgcgacgctctaaaggaagt

SEQ ID NO: 122 - DNA, 20 bp, Artificial Sequence
  Primer
ctctcagaccaggcccagca

SEQ ID NO: 123 - DNA, 20 bp, Artificial Sequence
  Primer
gctgaggcaaagcgactcca

SEQ ID NO: 124 - DNA, 22 bp, Artificial Sequence
  Primer
ctctaaaggaagtgacctttag

SEQ ID NO: 125 - DNA, 20 bp, Artificial Sequence
  Primer
ggctgttactctcagaccag

SEQ ID NO: 126 - DNA, 21 bp, Artificial Sequence
  Primer
aacctaccgactgacctgcat

SEQ ID NO: 127 - DNA, 21 bp, Artificial Sequence
  Primer
cctgcatgacgtaggtccact

SEQ ID NO: 128 - DNA, 20 bp, Artificial Sequence
  Primer
gggtcagatccgacgtaaag

SEQ ID NO: 129 - DNA, 19 bp, Artificial Sequence
  Primer
gcgtgttcccagccgctag

SEQ ID NO: 130 - DNA, 20 bp, Artificial Sequence
  Primer
gggattggccgagtcaggtc

SEQ ID NO: 131 - DNA, 20 bp, Artificial Sequence
  Primer
acagagctgcctgctggagc

SEQ ID NO: 132 - DNA, 19 bp, Artificial Sequence
  Primer
cggcaagagctcggtgctc

SEQ ID NO: 133 - DNA, 21 bp, Artificial Sequence
  Primer
agaacttcgtgggcaggtaag

SEQ ID NO: 134 - DNA, 21 bp, Artificial Sequence
  Primer
cgtctgcaggaccgcgttttc

SEQ ID NO: 135 - DNA, 19 bp, Artificial Sequence
  Primer
agctgatcccgctggtgaa

SEQ ID NO: 136 - DNA, 22 bp, Artificial Sequence
  Primer
aatggctttgtatcgcacgatg

SEQ ID NO: 137 - DNA, 20 bp, Artificial Sequence
  Primer
ccactgccgcatccttactc

SEQ ID NO: 138 - DNA, 20 bp, Artificial Sequence
  Primer
cctggtccatccaccctctg

SEQ ID NO: 139 - DNA, 19 bp, Artificial Sequence
  Primer
tgcccgtccacgttccaac

SEQ ID NO: 140 - DNA, 19 bp, Artificial Sequence
  Primer
cacggacaccgccactctg

SEQ ID NO: 141 - DNA, 21 bp, Artificial Sequence
  Primer
gagcattggcacccctgattc

SEQ ID NO: 142 - DNA, 21 bp, Artificial Sequence
  Primer
cttacccgtggtttctgcctg

SEQ ID NO: 143 - DNA, 21 bp, Artificial Sequence
  Primer
agagcattggcacccctgatt

SEQ ID NO: 144 - DNA, 22 bp, Artificial Sequence
  Primer
acttctcttacccgtggtttct

SEQ ID NO: 145 - DNA, 19 bp, Artificial Sequence
  Primer
ctggggcctacgcgaagct

SEQ ID NO: 146 - DNA, 25 bp, Artificial Sequence
  Primer
ctctaaaagtgttacaaacattaag

SEQ ID NO: 147 - DNA, 20 bp, Artificial Sequence
  Primer
tggaatcgtgcccggatcag

SEQ ID NO: 148 - DNA, 26 bp, Artificial Sequence
  Primer
tttttggaacgttaaataatttccta

SEQ ID NO: 149 - DNA, 22 bp, Artificial Sequence
  Primer
cctcagtttcctcaaaaggaat

SEQ ID NO: 150 - DNA, 20 bp, Artificial Sequence
  Primer
cgtgcccggatcagagcaag

SEQ ID NO: 151 - DNA, 20 bp, Artificial Sequence
  Primer
gcctggaatcgtgcccggat

SEQ ID NO: 152 - DNA, 23 bp, Artificial Sequence
  Primer
tccaaggaagactaaaaacccag

SEQ ID NO: 153 - DNA, 21 bp, Artificial Sequence
  Primer
taaaaacccaggccgggaagc

SEQ ID NO: 154 - DNA, 22 bp, Artificial Sequence
  Primer
tggtttgttccaaggagtacag

SEQ ID NO: 155 - DNA, 23 bp, Artificial Sequence
  Primer
agtacagatagccttttcaaaag

SEQ ID NO: 156 - DNA, 23 bp, Artificial Sequence
  Primer
agcaaggtgaagactaacttttc

SEQ ID NO: 157 - DNA, 23 bp, Artificial Sequence
  Primer
cttgtacagaatcatcaggctaa

SEQ ID NO: 158 - DNA, 25 bp, Artificial Sequence
  Primer
gtccttggagacatctgagagattc

SEQ ID NO: 159 - DNA, 20 bp, Artificial Sequence
  Primer
gacatctgagagattccggg

SEQ ID NO: 160 - DNA, 22 bp, Artificial Sequence
  Primer
caaagaaagcaaggtgaagact

SEQ ID NO: 161 - DNA, 24 bp, Artificial Sequence
  Primer
cagtccttggagacatctgagaga

SEQ ID NO: 162 - DNA, 23 bp, Artificial Sequence
  Primer
tgaagtgaactattccttaggtg

SEQ ID NO: 163 - DNA, 23 bp, Artificial Sequence
  Primer
gtctccaaggactgaaataatgc

SEQ ID NO: 164 - DNA, 28 bp, Artificial Sequence
  Primer
gagtagcaaaaaatagctgaagtgaact

SEQ ID NO: 165 - DNA, 23 bp, Artificial Sequence
  Primer
tgacaaccaatgagtagcaaaaa

SEQ ID NO: 166 - DNA, 20 bp, Artificial Sequence
  Primer
gttgtcagtgtggccagaga

SEQ ID NO: 167 - DNA, 21 bp, Artificial Sequence
  Primer
tgttgtcagtgtggccagaga